European Patent Specification EP 3 597 747 B1, published March 15, 2023. Title: Mouse Fc-gamma-RII-specific Fc antibody. Applicant: CHUGAI SEIYAKU KABUSHIKI KAISHA. The sequence listing filed with the application follows.

SEQUENCE LISTING (47 sequences)

SEQ ID NO: 1 - protein, 119 aa, Artificial Sequence
  an artificially synthesized sequence
QVQLQESGPGLVKPSETLSLTCAVSGHSISHDHAWSWVRQPPGEGLEWIGFISYSGITNYNPSLQGRVTISRDNSKNTLYLQMNSLRAEDTAVYYCARSLARTTAMDYWGEGTLVTVSS

SEQ ID NO: 2 - protein, 214 aa, Artificial Sequence [sequence omitted]

SEQ ID NO: 3 - protein, 330 aa, Homo sapiens [sequence omitted]

SEQ ID NO: 4 - protein, 324 aa, Mus musculus
AKTTPPSVYPLAPGSAAQTNSMVTLGCLVKGYFPEPVTVTWNSGSLSSGVHTFPAVLQSDLYTLSSSVTVPSSTWPSETVTCNVAHPASSTKVDKKIVPRDCGCKPCICTVPEVSSVFIFPPKPKDVLTITLTPKVTCVVVDISKDDPEVQFSWFVDDVEVHTAQTQPREEQFNSTFRSVSELPIMHQDWLNGKEFKCRVNSAAFPAPIEKTISKTKGRPKAPQVYTIPPPKEQMAKDKVSLTCMITDFFPEDITVEWQWNGQPAENYKNTQPIMDTDGSYFVYSKLNVQKSNWEAGNTFTCSVLHEGLHNHHTEKSLSHSPGK

SEQ ID NO: 5 - protein, 324 aa, Artificial Sequence
  an artificially synthesized sequence
AKTTPPSVYPLAPGSAAQTNSMVTLGCLVKGYFPEPVTVTWNSGSLSSGVHTFPAVLQSDLYTLSSSVTVPSSTWPSETVTCNVAHPASSTKVDKKIVPRDCGCKPCICETYEVEDVFIFPPKPKDVLTITLTPKVTCVVVDISKDDPEVQFSWFVDDVEVHTAQTQPREEQFNSTFRSVSELPIMHQDWLNGKEFKCRVNSAAFPAPIEKTISKTKGRPKAPQVYTIPPPKEQMAKDKVSLTCMITDFFPEDITVEWQWNGQPAENYKNTQPIMDTDGSYFVYSKLNVQKSNWEAGNTFTCSVLHEGLHNHHTEKSLSHSPGK

SEQ ID NO: 6 - protein, 324 aa, Artificial Sequence
  an artificially synthesized sequence
AKTTPPSVYPLAPGSAAQTNSMVTLGCLVKGYFPEPVTVTWNSGSLSSGVHTFPAVLQSDLYTLSSSVTVPSSTWPSETVTCNVAHPASSTKVDKKIVPRDCGCKPCICEPNEVEDVFIFPPKPKDVLTITLTPKVTCVVVDISKDDPEVQFSWFVDDVEVHTAQTQPREEQFNSTFRSVSELPIMHQDWLNGKEFKCRVNSAAFPAPIEKTISKTKGRPKAPQVYTIPPPKEQMAKDKVSLTCMITDFFPEDITVEWQWNGQPAENYKNTQPIMDTDGSYFVYSKLNVQKSNWEAGNTFTCSVLHEGLHNHHTEKSLSHSPGK

SEQ ID NO: 7 - protein, 443 aa, Artificial Sequence
  an artificially synthesized sequence
QVQLQESGPGLVKPSETLSLTCAVSGHSISHDHAWSWVRQPPGEGLEWIGFISYSGITNYNPSLQGRVTISRDNSKNTLYLQMNSLRAEDTAVYYCARSLARTTAMDYWGEGTLVTVSSAKTTPPSVYPLAPGSAAQTNSMVTLGCLVKGYFPEPVTVTWNSGSLSSGVHTFPAVLQSDLYTLSSSVTVPSSTWPSETVTCNVAHPASSTKVDKKIVPRDCGCKPCICTVPEVSSVFIFPPKPKDVLTITLTPKVTCVVVDISKDDPEVQFSWFVDDVEVHTAQTQPREEQFNSTFRSVSELPIMHQDWLNGKEFKCRVNSAAFPAPIEKTISKTKGRPKAPQVYTIPPPKEQMAKDKVSLTCMITDFFPEDITVEWQWNGQPAENYKNTQPIMDTDGSYFVYSKLNVQKSNWEAGNTFTCSVLHEGLHNHHTEKSLSHSPGK

SEQ ID NO: 8 - protein, 443 aa, Artificial Sequence
  an artificially synthesized sequence
QVQLQESGPGLVKPSETLSLTCAVSGHSISHDHAWSWVRQPPGEGLEWIGFISYSGITNYNPSLQGRVTISRDNSKNTLYLQMNSLRAEDTAVYYCARSLARTTAMDYWGEGTLVTVSSAKTTPPSVYPLAPGSAAQTNSMVTLGCLVKGYFPEPVTVTWNSGSLSSGVHTFPAVLQSDLYTLSSSVTVPSSTWPSETVTCNVAHPASSTKVDKKIVPRDCGCKPCICEANEVEDVFIFPPKPKDVLTITLTPKVTCVVVDISKDDPEVQFSWFVDDVEVHTAQTQPREEQFNSTFRSVSELPIMHQDWLNGKEFKCRVNSAAFPAPIEKTISKTKGRPKAPQVYTIPPPKEQMAKDKVSLTCMITDFFPEDITVEWQWNGQPAENYKNTQPIMDTDGSYFVYSKLNVQKSNWEAGNTFTCSVLHEGLHNHHTEKSLSHSPGK

SEQ ID NO: 9 - protein, 443 aa, Artificial Sequence
  an artificially synthesized sequence
QVQLQESGPGLVKPSETLSLTCAVSGHSISHDHAWSWVRQPPGEGLEWIGFISYSGITNYNPSLQGRVTISRDNSKNTLYLQMNSLRAEDTAVYYCARSLARTTAMDYWGEGTLVTVSSAKTTPPSVYPLAPGSAAQTNSMVTLGCLVKGYFPEPVTVTWNSGSLSSGVHTFPAVLQSDLYTLSSSVTVPSSTWPSETVTCNVAHPASSTKVDKKIVPRDCGCKPCICTVPEVSDVFIFPPKPKDVLTITLTPKVTCVVVDISKDDPEVQFSWFVDDVEVHTAQTQPREEQFNSTFRSVSELPIMHQDWLNGKEFKCRVNSADFPAPIEKTISKTKGRPKAPQVYTIPPPKEQMAKDKVSLTCMITDFFPEDITVEWQWNGQPAENYKNTQPIMDTDGSYFVYSKLNVQKSNWEAGNTFTCSVLHEGLHNHHTEKSLSHSPGK

SEQ ID NO: 10 - DNA, 1125 bp, Homo sapiens
atgtggttcttgacaactctgctcctttgggttccagttgatgggcaagtggacaccacaaaggcagtgatcactttgcagcctccatgggtcagcgtgttccaagaggaaaccgtaaccttgcactgtgaggtgctccatctgcctgggagcagctctacacagtggtttctcaatggcacagccactcagacctcgacccccagctacagaatcacctctgccagtgtcaatgacagtggtgaatacaggtgccagagaggtctctcagggcgaagtgaccccatacagctggaaatccacagaggctggctactactgcaggtctccagcagagtcttcacggaaggagaacctctggccttgaggtgtcatgcgtggaaggataagctggtgtacaatgtgctttactatcgaaatggcaaagcctttaagtttttccactggaattctaacctcaccattctgaaaaccaacataagtcacaatggcacctaccattgctcaggcatgggaaagcatcgctacacatcagcaggaatatctgtcactgtgaaagagctatttccagctccagtgctgaatgcatctgtgacatccccactcctggaggggaatctggtcaccctgagctgtgaaacaaagttgctcttgcagaggcctggtttgcagctttacttctccttctacatgggcagcaagaccctgcgaggcaggaacacatcctctgaataccaaatactaactgctagaagagaagactctgggttatactggtgcgaggctgccacagaggatggaaatgtccttaagcgcagccctgagttggagcttcaagtgcttggcctccagttaccaactcctgtctggtttcatgtccttttctatctggcagtgggaataatgtttttagtgaacactgttctctgggtgacaatacgtaaagaactgaaaagaaagaaaaagtgggatttagaaatctctttggattctggtcatgagaagaaggtaatttccagccttcaagaagacagacatttagaagaagagctgaaatgtcaggaacaaaaagaagaacagctgcaggaaggggtgcaccggaaggagccccagggggccacgtag

SEQ ID NO: 11 - protein, 374 aa, Homo sapiens
MWFLTTLLLWVPVDGQVDTTKAVITLQPPWVSVFQEETVTLHCEVLHLPGSSSTQWFLNGTATQTSTPSYRITSASVNDSGEYRCQRGLSGRSDPIQLEIHRGWLLLQVSSRVFTEGEPLALRCHAWKDKLVYNVLYYRNGKAFKFFHWNSNLTILKTNISHNGTYHCSGMGKHRYTSAGISVTVKELFPAPVLNASVTSPLLEGNLVTLSCETKLLLQRPGLQLYFSFYMGSKTLRGRNTSSEYQILTARREDSGLYWCEAATEDGNVLKRSPELELQVLGLQLPTPVWFHVLFYLAVGIMFLVNTVLWVTIRKELKRKKKWDLEISLDSGHEKKVISSLQEDRHLEEELKCQEQKEEQLQEGVHRKEPQGAT

SEQ ID NO: 12 - DNA, 951 bp, Homo sapiens
atgactatggagacccaaatgtctcagaatgtatgtcccagaaacctgtggctgcttcaaccattgacagttttgctgctgctggcttctgcagacagtcaagctgctcccccaaaggctgtgctgaaacttgagcccccgtggatcaacgtgctccaggaggactctgtgactctgacatgccagggggctcgcagccctgagagcgactccattcagtggttccacaatgggaatctcattcccacccacacgcagcccagctacaggttcaaggccaacaacaatgacagcggggagtacacgtgccagactggccagaccagcctcagcgaccctgtgcatctgactgtgctttccgaatggctggtgctccagacccctcacctggagttccaggagggagaaaccatcatgctgaggtgccacagctggaaggacaagcctctggtcaaggtcacattcttccagaatggaaaatcccagaaattctcccatttggatcccaccttctccatcccacaagcaaaccacagtcacagtggtgattaccactgcacaggaaacataggctacacgctgttctcatccaagcctgtgaccatcactgtccaagtgcccagcatgggcagctcttcaccaatgggggtcattgtggctgtggtcattgcgactgctgtagcagccattgttgctgctgtagtggccttgatctactgcaggaaaaagcggatttcagccaattccactgatcctgtgaaggctgcccaatttgagccacctggacgtcaaatgattgccatcagaaagagacaacttgaagaaaccaacaatgactatgaaacagctgacggcggctacatgactctgaaccccagggcacctactgacgatgataaaaacatctacctgactcttcctcccaacgaccatgtcaacagtaataactaa

SEQ ID NO: 13 - protein, 316 aa, Homo sapiens
MTMETQMSQNVCPRNLWLLQPLTVLLLLASADSQAAPPKAVLKLEPPWINVLQEDSVTLTCQGARSPESDSIQWFHNGNLIPTHTQPSYRFKANNNDSGEYTCQTGQTSLSDPVHLTVLSEWLVLQTPHLEFQEGETIMLRCHSWKDKPLVKVTFFQNGKSQKFSHLDPTFSIPQANHSHSGDYHCTGNIGYTLFSSKPVTITVQVPSMGSSSPMGVIVAVVIATAVAAIVAAVVALIYCRKKRISANSTDPVKAAQFEPPGRQMIAIRKRQLEETNNDYETADGGYMTLNPRAPTDDDKNIYLTLPPNDHVNSNN

SEQ ID NO: 14 - DNA, 876 bp, Homo sapiens
atgggaatcctgtcattcttacctgtccttgccactgagagtgactgggctgactgcaagtccccccagccttggggtcatatgcttctgtggacagctgtgctattcctggctcctgttgctgggacacctgcagctcccccaaaggctgtgctgaaactcgagccccagtggatcaacgtgctccaggaggactctgtgactctgacatgccgggggactcacagccctgagagcgactccattcagtggttccacaatgggaatctcattcccacccacacgcagcccagctacaggttcaaggccaacaacaatgacagcggggagtacacgtgccagactggccagaccagcctcagcgaccctgtgcatctgactgtgctttctgagtggctggtgctccagacccctcacctggagttccaggagggagaaaccatcgtgctgaggtgccacagctggaaggacaagcctctggtcaaggtcacattcttccagaatggaaaatccaagaaattttcccgttcggatcccaacttctccatcccacaagcaaaccacagtcacagtggtgattaccactgcacaggaaacataggctacacgctgtactcatccaagcctgtgaccatcactgtccaagctcccagctcttcaccgatggggatcattgtggctgtggtcactgggattgctgtagcggccattgttgctgctgtagtggccttgatctactgcaggaaaaagcggatttcagccaatcccactaatcctgatgaggctgacaaagttggggctgagaacacaatcacctattcacttctcatgcacccggatgctctggaagagcctgatgaccagaaccgtatttag

SEQ ID NO: 15 - protein, 291 aa, Homo sapiens
MGILSFLPVLATESDWADCKSPQPWGHMLLWTAVLFLAPVAGTPAAPPKAVLKLEPQWINVLQEDSVTLTCRGTHSPESDSIQWFHNGNLIPTHTQPSYRFKANNNDSGEYTCQTGQTSLSDPVHLTVLSEWLVLQTPHLEFQEGETIVLRCHSWKDKPLVKVTFFQNGKSKKFSRSDPNFSIPQANHSHSGDYHCTGNIGYTLYSSKPVTITVQAPSSSPMGIIVAVVTGIAVAAIVAAVVALIYCRKKRISANPTNPDEADKVGAENTITYSLLMHPDALEEPDDQNRI

SEQ ID NO: 16 - DNA, 765 bp, Homo sapiens
atgtggcagctgctcctcccaactgctctgctacttctagtttcagctggcatgcggactgaagatctcccaaaggctgtggtgttcctggagcctcaatggtacagggtgctcgagaaggacagtgtgactctgaagtgccagggagcctactcccctgaggacaattccacacagtggtttcacaatgagagcctcatctcaagccaggcctcgagctacttcattgacgctgccacagttgacgacagtggagagtacaggtgccagacaaacctctccaccctcagtgacccggtgcagctagaagtccatatcggctggctgttgctccaggcccctcggtgggtgttcaaggaggaagaccctattcacctgaggtgtcacagctggaagaacactgctctgcataaggtcacatatttacagaatggcaaaggcaggaagtattttcatcataattctgacttctacattccaaaagccacactcaaagacagcggctcctacttctgcagggggcttgttgggagtaaaaatgtgtcttcagagactgtgaacatcaccatcactcaaggtttgtcagtgtcaaccatctcatcattctttccacctgggtaccaagtctctttctgcttggtgatggtactcctttttgcagtggacacaggactatatttctctgtgaagacaaacattcgaagctcaacaagagactggaaggaccataaatttaaatggagaaaggaccctcaagacaaatga

SEQ ID NO: 17 - protein, 254 aa, Homo sapiens [sequence omitted]

SEQ ID NO: 18 - DNA, 702 bp, Homo sapiens
atgtggcagctgctcctcccaactgctctgctacttctagtttcagctggcatgcggactgaagatctcccaaaggctgtggtgttcctggagcctcaatggtacagcgtgcttgagaaggacagtgtgactctgaagtgccagggagcctactcccctgaggacaattccacacagtggtttcacaatgagagcctcatctcaagccaggcctcgagctacttcattgacgctgccacagtcaacgacagtggagagtacaggtgccagacaaacctctccaccctcagtgacccggtgcagctagaagtccatatcggctggctgttgctccaggcccctcggtgggtgttcaaggaggaagaccctattcacctgaggtgtcacagctggaagaacactgctctgcataaggtcacatatttacagaatggcaaagacaggaagtattttcatcataattctgacttccacattccaaaagccacactcaaagatagcggctcctacttctgcagggggcttgttgggagtaaaaatgtgtcttcagagactgtgaacatcaccatcactcaaggtttggcagtgtcaaccatctcatcattctctccacctgggtaccaagtctctttctgcttggtgatggtactcctttttgcagtggacacaggactatatttctctgtgaagacaaacatttga

SEQ ID NO: 19 - protein, 233 aa, Homo sapiens
MWQLLLPTALLLLVSAGMRTEDLPKAVVFLEPQWYSVLEKDSVTLKCQGAYSPEDNSTQWFHNESLISSQASSYFIDAATVNDSGEYRCQTNLSTLSDPVQLEVHIGWLLLQAPRWVFKEEDPIHLRCHSWKNTALHKVTYLQNGKDRKYFHHNSDFHIPKATLKDSGSYFCRGLVGSKNVSSETVNITITQGLAVSTISSFSPPGYQVSFCLVMVLLFAVDTGLYFSVKTNI

SEQ ID NO: 20 - protein, 404 aa, Mus musculus
MILTSFGDDMWLLTTLLLWVPVGGEVVNATKAVITLQPPWVSIFQKENVTLWCEGPHLPGDSSTQWFINGTAVQISTPSYSIPEASFQDSGEYRCQIGSSMPSDPVQLQIHNDWLLLQASRRVLTEGEPLALRCHGWKNKLVYNVVFYRNGKSFQFSSDSEVAILKTNLSHSGIYHCSGTGRHRYTSAGVSITVKELFTTPVLRASVSSPFPEGSLVTLNCETNLLLQRPGLQLHFSFYVGSKILEYRNTSSEYHIARAEREDAGFYWCEVATEDSSVLKRSPELELQVLGPQSSAPVWFHILFYLSVGIMFSLNTVLYVKIHRLQREKKYNLEVPLVSEQGKKANSFQQVRSDGVYEEVTATASQTTPKEAPDGPRSSVGDCGPEQPEPLPPSDSTGAQTSQS

SEQ ID NO: 21 - protein, 293 aa, Mus musculus
MGILPFLLIPMESNWTVHVFSRTLCHMLLWTAVLNLAAGTHDLPKAVVKLEPPWIQVLKEDTVTLTCEGTHNPGNSSTQWFHNGRSIRSQVQASYTFKATVNDSGEYRCQMEQTRLSDPVDLGVISDWLLLQTPQLVFLEGETITLRCHSWRNKLLNRISFFHNEKSVRYHHYSSNFSIPKANHSHSGDYYCKGSLGRTLHQSKPVTITVQGPKSSRSLPVLTIVAAVTGIAVAAIVIILVSLVYLKKKQVPDNPPDLEEAAKTEAENTITYSLLKHPEALDEETEHDYQNHI

SEQ ID NO: 22 - protein, 267 aa, Mus musculus
MTLDTQMFQNAHSGSQWLLPPLTILLLFAFADRQSAALPKAVVKLDPPWIQVLKEDMVTLMCEGTHNPGNSSTQWFHNWSSIRSQVQSSYTFKATVNDSGEYRCQMEQTRLSDPVDLGVISDWLLLQTPQRVFLEGETITLRCHSWRNKLLNRISFFHNEKSVRYHHYKSNFSIPKANHSHSGDYYCKGSLGSTQHQSKPVTITVQDPATTSSISLVWYHTAFSLVMCLLFAVDTGLYFYVRRNLQTPRDYWRKSLSIRKHQAPQDK

SEQ ID NO: 23 - protein, 249 aa, Mus musculus
MWQLLLPTALVLTAFSGIQAGLQKAVVNLDPKWVRVLEEDSVTLRCQGTFSPEDNSIKWFHNESLIPHQDANYVIQSARVKDSGMYRCQTALSTISDPVQLEVHMGWLLLQTTKWLFQEGDPIHLRCHSWQNRPVRKVTYLQNGKGKKYFHENSELLIPKATHNDSGSYFCRGLIGHNNKSSASFRISLGDPGSPSMFPPWHQITFCLLIGLLFAIDTVLYFSVRRGLQSPVADYEEPKIQWSKEPQDK

SEQ ID NO: 24 - protein, 324 aa, Mus musculus; identical to SEQ ID NO: 4

SEQ ID NO: 25 - protein, 330 aa, Mus musculus
AKTTAPSVYPLAPVCGDTTGSSVTLGCLVKGYFPEPVTLTWNSGSLSSGVHTFPAVLQSDLYTLSSSVTVTSSTWPSQSITCNVAHPASSTKVDKKIEPRGPTIKPCPPCKCPAPNLLGGPSVFIFPPKIKDVLMISLSPIVTCVVVDVSEDDPDVQISWFVNNVEVHTAQTQTHREDYNSTLRVVSALPIQHQDWMSGKEFKCKVNNKDLPAPIERTISKPKGSVRAPQVYVLPPPEEEMTKKQVTLTCMVTDFMPEDIYVEWTNNGKTELNYKNTEPVLDSDGSYFMYSKLRVEKKNWVERNSYSCSVVHEGLHNHHTTKSFSRTPGK

SEQ ID NO: 26 - protein, 336 aa, Mus musculus
AKTTPPSVYPLAPGCGDTTGSSVTSGCLVKGYFPEPVTVTWNSGSLSSSVHTFPALLQSGLYTMSSSVTVPSSTWPSQTVTCSVAHPASSTTVDKKLEPSGPISTINPCPPCKECHKCPAPNLEGGPSVFIFPPNIKDVLMISLTPKVTCVVVDVSEDDPDVQISWFVNNVEVHTAQTQTHREDYNSTIRVVSTLPIQHQDWMSGKEFKCKVNNKDLPSPIERTISKIKGLVRAPQVYTLPPPAEQLSRKDVSLTCLVVGFNPGDISVEWTSNGHTEENYKDTAPVLDSDGSYFIYSKLNMKTSKWEKTDSFSCNVRHEGLKNYYLKKTISRSPGK

SEQ ID NO: 27 - protein, 330 aa, Mus musculus
ATTTAPSVYPLVPGCSDTSGSSVTLGCLVKGYFPEPVTVKWNYGALSSGVRTVSSVLQSGFYSLSSLVTVPSSTWPSQTVICNVAHPASKTELIKRIEPRIPKPSTPPGSSCPPGNILGGPSVFIFPPKPKDALMISLTPKVTCVVVDVSEDDPDVHVSWFVDNKEVHTAWTQPREAQYNSTFRVVSALPIQHQDWMRGKEFKCKVNNKALPAPIERTISKPKGRAQTPQVYTIPPPREQMSKKKVSLTCLVTNFFSEAISVEWERNGELEQDYKNTPPILDSDGTYFLYSKLTVDTDSWLQGEIFTCSVVHEALHNHHTQKNLSRSPGK

SEQ ID NO: 28 - protein, 330 aa, Homo sapiens [sequence omitted]

SEQ ID NO: 29 - protein, 326 aa, Homo sapiens
ASTKGPSVFPLAPCSRSTSESTAALGCLVKDYFPEPVTVSWNSGALTSGVHTFPAVLQSSGLYSLSSVVTVPSSNFGTQTYTCNVDHKPSNTKVDKTVERKCCVECPPCPAPPVAGPSVFLFPPKPKDTLMISRTPEVTCVVVDVSHEDPEVQFNWYVDGVEVHNAKTKPREEQFNSTFRVVSVLTVVHQDWLNGKEYKCKVSNKGLPAPIEKTISKTKGQPREPQVYTLPPSREEMTKNQVSLTCLVKGFYPSDIAVEWESNGQPENNYKTTPPMLDSDGSFFLYSKLTVDKSRWQQGNVFSCSVMHEALHNHYTQKSLSLSPGK

SEQ ID NO: 30 - protein, 377 aa, Homo sapiens
ASTKGPSVFPLAPCSRSTSGGTAALGCLVKDYFPEPVTVSWNSGALTSGVHTFPAVLQSSGLYSLSSVVTVPSSSLGTQTYTCNVNHKPSNTKVDKRVELKTPLGDTTHTCPRCPEPKSCDTPPPCPRCPEPKSCDTPPPCPRCPEPKSCDTPPPCPRCPAPELLGGPSVFLFPPKPKDTLMISRTPEVTCVVVDVSHEDPEVQFKWYVDGVEVHNAKTKPREEQYNSTFRVVSVLTVLHQDWLNGKEYKCKVSNKALPAPIEKTISKTKGQPREPQVYTLPPSREEMTKNQVSLTCLVKGFYPSDIAVEWESSGQPENNYNTTPPMLDSDGSFFLYSKLTVDKSRWQQGNIFSCSVMHEALHNRFTQKSLSLSPGK

SEQ ID NO: 31 - protein, 327 aa, Homo sapiens
ASTKGPSVFPLAPCSRSTSESTAALGCLVKDYFPEPVTVSWNSGALTSGVHTFPAVLQSSGLYSLSSVVTVPSSSLGTKTYTCNVDHKPSNTKVDKRVESKYGPPCPSCPAPEFLGGPSVFLFPPKPKDTLMISRTPEVTCVVVDVSQEDPEVQFNWYVDGVEVHNAKTKPREEQFNSTYRVVSVLTVLHQDWLNGKEYKCKVSNKGLPSSIEKTISKAKGQPREPQVYTLPPSQEEMTKNQVSLTCLVKGFYPSDIAVEWESNGQPENNYKTTPPVLDSDGSFFLYSRLTVDKSRWQEGNVFSCSVMHEALHNHYTQKSLSLSLGK

SEQ ID NO: 32 - protein, 214 aa, Artificial Sequence
  an artificially synthesized sequence
DIQMTQSPSSLSASVGDSVTITCQASTDISSHLNWYQQKPGKAPELLIYYGSHLLSGVPSRFSGSGSGTDFTFTISSLEAEDAATYYCGQGNRLPYTFGQGTKVEIERADAAPTVSIFPPSSEQLTSGGASVVCFLNNFYPKDINVKWKIDGSERQNGVLNSWTDQDSKDSTYSMSSTLTLTKDEYERHNSYTCEATHKTSTSPIVKSFNRNEC

SEQ ID NO: 33 - DNA, 1215 bp, Mus musculus
atgattcttaccagctttggagatgacatgtggcttctaacaactctgctactttgggttccagtcggtggggaagtggttaatgccaccaaggctgtgatcaccttgcagcctccatgggtcagtattttccagaaggaaaatgtcactttatggtgtgaggggcctcacctgcctggagacagttccacacaatggtttatcaacggaacagccgttcagatctccacgcctagttatagcatcccagaggccagttttcaggacagtggcgaatacaggtgtcagataggttcctcaatgccaagtgaccctgtgcagttgcaaatccacaatgattggctgctactccaggcctcccgcagagtcctcacagaaggagaacccctggccttgaggtgtcacggatggaagaataaactggtgtacaatgtggttttctatagaaatggaaaatcctttcagttttcttcagattcggaggtcgccattctgaaaaccaacctgagtcacagcggcatctaccactgctcaggcacgggaagacaccgctacacatctgcaggagtgtccatcacggtgaaagagctgtttaccacgccagtgctgagagcatccgtgtcatctcccttcccggaggggagtctggtcaccctgaactgtgagacgaatttgctcctgcagagacccggcttacagcttcacttctccttctacgtgggcagcaagatcctggagtacaggaacacatcctcagagtaccatatagcaagggcggaaagagaagatgctggattctactggtgtgaggtagccacggaggacagcagtgtccttaagcgcagccctgagttggagctccaagtgcttggtccccagtcatcagctcctgtctggtttcacatcctgttttatctgtcagtgggaataatgttttcgttgaacacggttctctatgtgaaaatacacaggctgcagagagagaagaaatacaacttagaagtccctttggtttctgagcagggaaagaaagcaaattcctttcagcaagttagaagcgatggcgtgtatgaagaagtaacagccactgcgagccagaccacaccaaaagaagcgcccgatggacctcgaagctcagtgggtgactgtggacccgagcagcctgaaccccttcctcccagtgacagtactggggcacaaacttcccaaagttga

SEQ ID NO: 34 - DNA, 882 bp, Mus musculus
atgggaatcctgccgttcctactgatccccatggagagcaactggactgtccatgtgttctcacggactttgtgccatatgctactgtggacagccgtgctaaatcttgctgctgggactcatgatcttccaaaggctgtggtcaaactcgagcccccgtggatccaggtgctcaaggaagacacggtgacactgacatgcgaagggacccacaaccctgggaactcttctacccagtggttccacaatgggaggtccatccggagccaggtccaagccagctacacgtttaaggccacagtcaatgacagtggagaatatcggtgtcaaatggagcagacccgcctcagcgaccctgtagatctgggagtgatttctgactggctgctgctccagacccctcagctggtgtttctggaaggggaaaccatcacgctaaggtgccatagctggaggaacaaactactgaacaggatctcgttcttccataatgaaaaatccgtgaggtatcatcactacagtagtaatttctctatcccaaaagccaaccacagtcacagtggggactactactgcaaaggaagtctaggaaggacactgcaccagtccaagcctgtcaccatcactgtccaagggcccaagtccagcaggtctttaccagtattgacaattgtggctgctgtcactgggattgctgtcgcagccattgttattatcctagtatccttggtctatctcaagaaaaagcaggttccagacaatcctcctgatctggaagaagctgccaaaactgaggctgagaatacgatcacctactcacttctcaagcatcccgaagccctggatgaagaaacagagcatgattaccagaaccacatttag

SEQ ID NO: 35 - DNA, 804 bp, Mus musculus
atgactttggacacccagatgtttcagaatgcacactctggaagccaatggctacttccaccactgacaattctgctgctgtttgcttttgcagacaggcagagtgcagctcttccgaaggctgtggtgaaactggaccccccatggatccaggtgctcaaggaagacatggtgacactgatgtgcgaagggacccacaaccctgggaactcttctactcagtggttccacaactggagttccatccggagccaggtccaatccagctacacgtttaaggccacagtcaatgacagtggagaatatcggtgtcaaatggagcagacccgcctcagcgaccctgtagatctgggagtgatttctgactggctgctgctccagacccctcagcgggtgtttctggaaggggaaaccatcacgctaaggtgccatagctggaggaacaaactactgaacaggatctcgttcttccataatgaaaaatccgtgaggtatcatcactacaaaagtaatttctctatcccaaaagccaaccacagtcacagtggggactactactgcaaaggaagtctaggaagtacacagcaccagtccaagcctgtcaccatcactgtccaagacccagcaactacatcctccatctctctagtctggtaccacactgctttctccctagtgatgtgcctcctgtttgcagtggacacgggcctttatttctatgtacggagaaatcttcaaaccccgagggattactggaggaagtccctgtcaatcagaaagcaccaggctcctcaagacaagtga

SEQ ID NO: 36 - DNA, 750 bp, Mus musculus
atgtggcagctactactaccaacagctctggtacttacagctttctctggcattcaagctggtctccaaaaggctgtggtgaacctagaccccaagtgggtcagggtgcttgaggaagacagcgtgaccctcagatgccaaggcactttctcccccgaggacaattctatcaagtggttccataacgaaagcctcatcccacaccaggatgccaactatgtcatccaaagtgccagagttaaggacagtggaatgtacaggtgccagacagccctctccacgatcagtgacccagtgcaactagaggtccatatgggctggctattgcttcagaccactaagtggctgttccaggagggggaccccattcatctgagatgccacagttggcaaaacagacctgtacggaaggtcacctatttacagaacggcaaaggcaagaagtatttccatgaaaattctgaattactcattccaaaagctacacacaatgacagtggctcctacttctgcagagggctcattggacacaacaacaaatcttcagcatcctttcgtataagcctaggcgatccagggtctccatccatgtttccaccgtggcatcaaatcacattctgcctgctgataggactcttgtttgcaatagacacagtgctgtatttctctgtgcggaggggtcttcaaagtcctgtggctgactatgaggaacccaagattcaatggagcaaggaacctcaggacaagtga

SEQ ID NO: 37 - protein, 324 aa, Artificial Sequence
  an artificially synthesized sequence
AKTTPPSVYPLAPGSAAQTNSMVTLGCLVKGYFPEPVTVTWNSGSLSSGVHTFPAVLQSDLYTLSSSVTVPSSTWPSETVTCNVAHPASSTKVDKKIVPRDCGCKPCICQPNEVEEVFIFPPKPKDVLTITLTPKVTCVVVDISKDDPEVQFSWFVDDVEVHTAQTQPREEQFNSTFRSVSELPIMHQDWLNGKEFKCRVNSAAFPAPIEKTISKTKGRPKAPQVYTIPPPKEQMAKDKVSLTCMITDFFPEDITVEWQWNGQPAENYKNTQPIMDTDGSYFVYSKLNVQKSNWEAGNTFTCSVLHEGLHNHHTEKSLSHSPGK

SEQ ID NO: 38 - protein, 324 aa, Artificial Sequence
  an artificially synthesized sequence
AKTTPPSVYPLAPGSAAQTNSMVTLGCLVKGYFPEPVTVTWNSGSLSSGVHTFPAVLQSDLYTLSSSVTVPSSTWPSETVTCNVAHPASSTKVDKKIVPRDCGCKPCICEPNEVEMVFIFPPKPKDVLTITLTPKVTCVVVDISKDDPEVQFSWFVDDVEVHTAQTQPREEQFNSTFRSVSELPIMHQDWLNGKEFKCRVNSAAFPAPIEKTISKTKGRPKAPQVYTIPPPKEQMAKDKVSLTCMITDFFPEDITVEWQWNGQPAENYKNTQPIMDTDGSYFVYSKLNVQKSNWEAGNTFTCSVLHEGLHNHHTEKSLSHSPGK

SEQ ID NO: 39 - protein, 324 aa, Artificial Sequence
  an artificially synthesized sequence
AKTTPPSVYPLAPGSAAQTNSMVTLGCLVKGYFPEPVTVTWNSGSLSSGVHTFPAVLQSDLYTLSSSVTVPSSTWPSETVTCNVAHPASSTKVDKKIVPRDCGCKPCICEPNEVELVFIFPPKPKDVLTITLTPKVTCVVVDISKDDPEVQFSWFVDDVEVHTAQTQPREEQFNSTFRSVSELPIMHQDWLNGKEFKCRVNSAAFPAPIEKTISKTKGRPKAPQVYTIPPPKEQMAKDKVSLTCMITDFFPEDITVEWQWNGQPAENYKNTQPIMDTDGSYFVYSKLNVQKSNWEAGNTFTCSVLHEGLHNHHTEKSLSHSPGK

SEQ ID NO: 40 - protein, 324 aa, Artificial Sequence
  an artificially synthesized sequence
AKTTPPSVYPLAPGSAAQTNSMVTLGCLVKGYFPEPVTVTWNSGSLSSGVHTFPAVLQSDLYTLSSSVTVPSSTWPSETVTCNVAHPASSTKVDKKIVPRDCGCKPCICEAYEVEDVFIFPPKPKDVLTITLTPKVTCVVVDISKDDPEVQFSWFVDDVEVHTAQTQPREEQFNSTFRSVSELPIMHQDWLNGKEFKCRVNSAAFPAPIEKTISKTKGRPKAPQVYTIPPPKEQMAKDKVSLTCMITDFFPEDITVEWQWNGQPAENYKNTQPIMDTDGSYFVYSKLNVQKSNWEAGNTFTCSVLHEGLHNHHTEKSLSHSPGK

SEQ ID NO: 41 - protein, 324 aa, Artificial Sequence
  an artificially synthesized sequence
AKTTPPSVYPLAPGSAAQTNSMVTLGCLVKGYFPEPVTVTWNSGSLSSGVHTFPAVLQSDLYTLSSSVTVPSSTWPSETVTCNVAHPASSTKVDKKIVPRDCGCKPCICEDYEVEDVFIFPPKPKDVLTITLTPKVTCVVVDISKDDPEVQFSWFVDDVEVHTAQTQPREEQFNSTFRSVSELPIMHQDWLNGKEFKCRVNSAAFPAPIEKTISKTKGRPKAPQVYTIPPPKEQMAKDKVSLTCMITDFFPEDITVEWQWNGQPAENYKNTQPIMDTDGSYFVYSKLNVQKSNWEAGNTFTCSVLHEGLHNHHTEKSLSHSPGK

SEQ ID NO: 42 - protein, 324 aa, Artificial Sequence
  an artificially synthesized sequence
AKTTPPSVYPLAPGSAAQTNSMVTLGCLVKGYFPEPVTVTWNSGSLSSGVHTFPAVLQSDLYTLSSSVTVPSSTWPSETVTCNVAHPASSTKVDKKIVPRDCGCKPCICENYEVEDVFIFPPKPKDVLTITLTPKVTCVVVDISKDDPEVQFSWFVDDVEVHTAQTQPREEQFNSTFRSVSELPIMHQDWLNGKEFKCRVNSAAFPAPIEKTISKTKGRPKAPQVYTIPPPKEQMAKDKVSLTCMITDFFPEDITVEWQWNGQPAENYKNTQPIMDTDGSYFVYSKLNVQKSNWEAGNTFTCSVLHEGLHNHHTEKSLSHSPGK

SEQ ID NO: 43 - protein, 324 aa, Artificial Sequence
  an artificially synthesized sequence
AKTTPPSVYPLAPGSAAQTNSMVTLGCLVKGYFPEPVTVTWNSGSLSSGVHTFPAVLQSDLYTLSSSVTVPSSTWPSETVTCNVAHPASSTKVDKKIVPRDCGCKPCICEVYEVEDVFIFPPKPKDVLTITLTPKVTCVVVDISKDDPEVQFSWFVDDVEVHTAQTQPREEQFNSTFRSVSELPIMHQDWLNGKEFKCRVNSAAFPAPIEKTISKTKGRPKAPQVYTIPPPKEQMAKDKVSLTCMITDFFPEDITVEWQWNGQPAENYKNTQPIMDTDGSYFVYSKLNVQKSNWEAGNTFTCSVLHEGLHNHHTEKSLSHSPGK

SEQ ID NO: 44 - protein, 324 aa, Artificial Sequence
  an artificially synthesized sequence
AKTTPPSVYPLAPGSAAQTNSMVTLGCLVKGYFPEPVTVTWNSGSLSSGVHTFPAVLQSDLYTLSSSVTVPSSTWPSETVTCNVAHPASSTKVDKKIVPRDCGCKPCICEPAEVEDVFIFPPKPKDVLTITLTPKVTCVVVDISKDDPEVQFSWFVDDVEVHTAQTQPREEQFNSTFRSVSELPIMHQDWLNGKEFKCRVNSAAFPAPIEKTISKTKGRPKAPQVYTIPPPKEQMAKDKVSLTCMITDFFPEDITVEWQWNGQPAENYKNTQPIMDTDGSYFVYSKLNVQKSNWEAGNTFTCSVLHEGLHNHHTEKSLSHSPGK

SEQ ID NO: 45 - protein, 324 aa, Artificial Sequence
  an artificially synthesized sequence
AKTTPPSVYPLAPGSAAQTNSMVTLGCLVKGYFPEPVTVTWNSGSLSSGVHTFPAVLQSDLYTLSSSVTVPSSTWPSETVTCNVAHPASSTKVDKKIVPRDCGCKPCICIPAEVEDVFIFPPKPKDVLTITLTPKVTCVVVDISKDDPEVQFSWFVDDVEVHTAQTQPREEQFNSTFRSVSELPIMHQDWLNGKEFKCRVNSAAFPAPIEKTISKTKGRPKAPQVYTIPPPKEQMAKDKVSLTCMITDFFPEDITVEWQWNGQPAENYKNTQPIMDTDGSYFVYSKLNVQKSNWEAGNTFTCSVLHEGLHNHHTEKSLSHSPGK

SEQ ID NO: 46 - protein, 324 aa, Artificial Sequence
  an artificially synthesized sequence
AKTTPPSVYPLAPGSAAQTNSMVTLGCLVKGYFPEPVTVTWNSGSLSSGVHTFPAVLQSDLYTLSSSVTVPSSTWPSETVTCNVAHPASSTKVDKKIVPRDCGCKPCICQPNEVEDVFIFPPKPKDVLTITLTPKVTCVVVDISKDDPEVQFSWFVDDVEVHTAQTQPREEQFNSTFRSVSELPIMHQDWLNGKEFKCRVNSAAFPAPIEKTISKTKGRPKAPQVYTIPPPKEQMAKDKVSLTCMITDFFPEDITVEWQWNGQPAENYKNTQPIMDTDGSYFVYSKLNVQKSNWEAGNTFTCSVLHEGLHNHHTEKSLSHSPGK

SEQ ID NO: 47 - protein, 324 aa, Artificial Sequence
  an artificially synthesized sequence
AKTTPPSVYPLAPGSAAQTNSMVTLGCLVKGYFPEPVTVTWNSGSLSSGVHTFPAVLQSDLYTLSSSVTVPSSTWPSETVTCNVAHPASSTKVDKKIVPRDCGCKPCICEPNEVEIVFIFPPKPKDVLTITLTPKVTCVVVDISKDDPEVQFSWFVDDVEVHTAQTQPREEQFNSTFRSVSELPIMHQDWLNGKEFKCRVNSAAFPAPIEKTISKTKGRPKAPQVYTIPPPKEQMAKDKVSLTCMITDFFPEDITVEWQWNGQPAENYKNTQPIMDTDGSYFVYSKLNVQKSNWEAGNTFTCSVLHEGLHNHHTEKSLSHSPGK